European Patent Specification EP 3 759 136 B1, published July 3, 2024. Title: Specific Binding Molecules for hTERT. Applicant: Oslo universitetssykehus HF. The sequence listing filed with the application follows.

SEQUENCE LISTING (68 sequences)

SEQ ID NO: 1 - protein, 12 aa, Homo sapiens
ALLTSRLRFIPK

SEQ ID NO: 2 - protein, 7 aa, Homo sapiens
TSDQSYG

SEQ ID NO: 3 - protein, 8 aa, Homo sapiens
QGSYDEQN

SEQ ID NO: 4 - protein, 15 aa, Homo sapiens
CAMREIYSSASKIIF

SEQ ID NO: 5 - protein, 5 aa, Homo sapiens
SGHTA

SEQ ID NO: 6 - protein, 6 aa, Homo sapiens
FQGNSA

SEQ ID NO: 7 - protein, 16 aa, Homo sapiens
CASSLGGGDHTDTQYF

SEQ ID NO: 8 - protein, 112 aa, Homo sapiens
ITQTQPGMFVQEKEAVTLDCTYDTSDQSYGLFWYKQPSSGEMIFLIYQGSYDEQNATEGRYSLNFQKARKSANLVISASQLGDSAMYFCAMREIYSSASKIIFGSGTRLSIR

SEQ ID NO: 9 - protein, 115 aa, Homo sapiens
AQKITQTQPGMFVQEKEAVTLDCTYDTSDQSYGLFWYKQPSSGEMIFLIYQGSYDEQNATEGRYSLNFQKARKSANLVISASQLGDSAMYFCAMREIYSSASKIIFGSGTRLSIR

SEQ ID NO: 10 - protein, 113 aa, Homo sapiens
VSQSPSNKVTEKGKDVELRCDPISGHTALYWYRQSLGQGLEFLIYFQGNSAPDKSGLPSDRFSAERTGGSVSTLTIQRTQQEDSAVYLCASSLGGGDHTDTQYFGPGTRLTVL

SEQ ID NO: 11 - protein, 116 aa, Homo sapiens
GAGVSQSPSNKVTEKGKDVELRCDPISGHTALYWYRQSLGQGLEFLIYFQGNSAPDKSGLPSDRFSAERTGGSVSTLTIQRTQQEDSAVYLCASSLGGGDHTDTQYFGPGTRLTVL

SEQ ID NO: 12 - protein, 142 aa, Homo sapiens
PNIQNPDPAVYQLRDSKSSDKSVCLFTDFDSQTNVSQSKDSDVYITDKTVLDMRSMDFKSNSAVAWSNKSDFACANAFNNSIIPEDTFFPSPESSCDVKLVEKSFETDTNLNFQNLSVIGFRILLLKVAGFNLLMTLRLWSS

SEQ ID NO: 13 - protein, 179 aa, Homo sapiens
EDLKNVFPPEVAVFEPSEAEISHTQKATLVCLATGFYPDHVELSWWVNGKEVHSGVSTDPQPLKEQPALNDSRYCLSSRLRVSATFWQNPRNHFRCQVQFYGLSENDEWTQDRAKPVTQIVSAEAWGRADCGFTSESYQQGVLSATILYEILLGKATLYAVLVSALVLMAMVKRKDSRG

SEQ ID NO: 14 - protein, 274 aa, Artificial Sequence
  Full length hTERT-TCR-1 alpha-chain with truncated variable region.
MSLSSLLKVVTASLWLGPGIITQTQPGMFVQEKEAVTLDCTYDTSDQSYGLFWYKQPSSGEMIFLIYQGSYDEQNATEGRYSLNFQKARKSANLVISASQLGDSAMYFCAMREIYSSASKIIFGSGTRLSIRPNIQNPDPAVYQLRDSKSSDKSVCLFTDFDSQTNVSQSKDSDVYITDKTVLDMRSMDFKSNSAVAWSNKSDFACANAFNNSIIPEDTFFPSPESSCDVKLVEKSFETDTNLNFQNLSVIGFRILLLKVAGFNLLMTLRLWSS

SEQ ID NO: 15 - protein, 277 aa, Homo sapiens
MSLSSLLKVVTASLWLGPGIAQKITQTQPGMFVQEKEAVTLDCTYDTSDQSYGLFWYKQPSSGEMIFLIYQGSYDEQNATEGRYSLNFQKARKSANLVISASQLGDSAMYFCAMREIYSSASKIIFGSGTRLSIRPNIQNPDPAVYQLRDSKSSDKSVCLFTDFDSQTNVSQSKDSDVYITDKTVLDMRSMDFKSNSAVAWSNKSDFACANAFNNSIIPEDTFFPSPESSCDVKLVEKSFETDTNLNFQNLSVIGFRILLLKVAGFNLLMTLRLWSS

SEQ ID NO: 16 - protein, 311 aa, Artificial Sequence
  Full length hTERT-TCR-1 beta-chain with truncated variable region
MGTRLLFWVAFCLLGADHTVSQSPSNKVTEKGKDVELRCDPISGHTALYWYRQSLGQGLEFLIYFQGNSAPDKSGLPSDRFSAERTGGSVSTLTIQRTQQEDSAVYLCASSLGGGDHTDTQYFGPGTRLTVLEDLKNVFPPEVAVFEPSEAEISHTQKATLVCLATGFYPDHVELSWWVNGKEVHSGVSTDPQPLKEQPALNDSRYCLSSRLRVSATFWQNPRNHFRCQVQFYGLSENDEWTQDRAKPVTQIVSAEAWGRADCGFTSESYQQGVLSATILYEILLGKATLYAVLVSALVLMAMVKRKDSRG

SEQ ID NO: 17 - protein, 314 aa, Homo sapiens
MGTRLLFWVAFCLLGADHTGAGVSQSPSNKVTEKGKDVELRCDPISGHTALYWYRQSLGQGLEFLIYFQGNSAPDKSGLPSDRFSAERTGGSVSTLTIQRTQQEDSAVYLCASSLGGGDHTDTQYFGPGTRLTVLEDLKNVFPPEVAVFEPSEAEISHTQKATLVCLATGFYPDHVELSWWVNGKEVHSGVSTDPQPLKEQPALNDSRYCLSSRLRVSATFWQNPRNHFRCQVQFYGLSENDEWTQDRAKPVTQIVSAEAWGRADCGFTSESYQQGVLSATILYEILLGKATLYAVLVSALVLMAMVKRKDSRG

SEQ ID NO: 18 - protein, 26 aa, Picornaviridae
RAKRGSGATNFSLLKQAGDVEENPGP

SEQ ID NO: 19 - protein, 611 aa, Artificial Sequence
  hTERT-TCR-1 scTCR with truncated variable regions
MSLSSLLKVVTASLWLGPGIITQTQPGMFVQEKEAVTLDCTYDTSDQSYGLFWYKQPSSGEMIFLIYQGSYDEQNATEGRYSLNFQKARKSANLVISASQLGDSAMYFCAMREIYSSASKIIFGSGTRLSIRPNIQNPDPAVYQLRDSKSSDKSVCLFTDFDSQTNVSQSKDSDVYITDKTVLDMRSMDFKSNSAVAWSNKSDFACANAFNNSIIPEDTFFPSPESSCDVKLVEKSFETDTNLNFQNLSVIGFRILLLKVAGFNLLMTLRLWSSRAKRGSGATNFSLLKQAGDVEENPGPMGTRLLFWVAFCLLGADHTVSQSPSNKVTEKGKDVELRCDPISGHTALYWYRQSLGQGLEFLIYFQGNSAPDKSGLPSDRFSAERTGGSVSTLTIQRTQQEDSAVYLCASSLGGGDHTDTQYFGPGTRLTVLEDLKNVFPPEVAVFEPSEAEISHTQKATLVCLATGFYPDHVELSWWVNGKEVHSGVSTDPQPLKEQPALNDSRYCLSSRLRVSATFWQNPRNHFRCQVQFYGLSENDEWTQDRAKPVTQIVSAEAWGRADCGFTSESYQQGVLSATILYEILLGKATLYAVLVSALVLMAMVKRKDSRG

SEQ ID NO: 20 - protein, 617 aa, Artificial Sequence
  hTERT-TCR-1 scTCR
MSLSSLLKVVTASLWLGPGIAQKITQTQPGMFVQEKEAVTLDCTYDTSDQSYGLFWYKQPSSGEMIFLIYQGSYDEQNATEGRYSLNFQKARKSANLVISASQLGDSAMYFCAMREIYSSASKIIFGSGTRLSIRPNIQNPDPAVYQLRDSKSSDKSVCLFTDFDSQTNVSQSKDSDVYITDKTVLDMRSMDFKSNSAVAWSNKSDFACANAFNNSIIPEDTFFPSPESSCDVKLVEKSFETDTNLNFQNLSVIGFRILLLKVAGFNLLMTLRLWSSRAKRGSGATNFSLLKQAGDVEENPGPMGTRLLFWVAFCLLGADHTGAGVSQSPSNKVTEKGKDVELRCDPISGHTALYWYRQSLGQGLEFLIYFQGNSAPDKSGLPSDRFSAERTGGSVSTLTIQRTQQEDSAVYLCASSLGGGDHTDTQYFGPGTRLTVLEDLKNVFPPEVAVFEPSEAEISHTQKATLVCLATGFYPDHVELSWWVNGKEVHSGVSTDPQPLKEQPALNDSRYCLSSRLRVSATFWQNPRNHFRCQVQFYGLSENDEWTQDRAKPVTQIVSAEAWGRADCGFTSESYQQGVLSATILYEILLGKATLYAVLVSALVLMAMVKRKDSRG

SEQ ID NO: 21 - protein, 96 aa, Artificial Sequence
  Soluble truncated human alpha-chain constant region containing cysteine substitution.
PNIQNPDPAVYQLRDSKSSDKSVCLFTDFDSQTNVSQSKDSDVYITDKCVLDMRSMDFKSNSAVAWSNKSDFACANAFNNSIIPEDTFFPSPESSC

SEQ ID NO: 22 - protein, 132 aa, Artificial Sequence
  Soluble truncated human beta-chain constant region containing cysteine substitution.
EDLKNVFPPEVAVFEPSEAEISHTQKATLVCLATGFYPDHVELSWWVNGKEVHSGVCTDPQPLKEQPALNDSRYCLSSRLRVSATFWQNPRNHFRCQVQFYGLSENDEWTQDRAKPVTQIVSAEAWGRADCG

SEQ ID NO: 23 - protein, 228 aa, Artificial Sequence
  Soluble hTERT-TCR-1 alpha-chain, with truncated variable region and truncated constant regioncontaining cysteine substitution.
MSLSSLLKVVTASLWLGPGIITQTQPGMFVQEKEAVTLDCTYDTSDQSYGLFWYKQPSSGEMIFLIYQGSYDEQNATEGRYSLNFQKARKSANLVISASQLGDSAMYFCAMREIYSSASKIIFGSGTRLSIRPNIQNPDPAVYQLRDSKSSDKSVCLFTDFDSQTNVSQSKDSDVYITDKCVLDMRSMDFKSNSAVAWSNKSDFACANAFNNSIIPEDTFFPSPESSC

SEQ ID NO: 24 - protein, 231 aa, Artificial Sequence
  Soluble hTERT-TCR-1 alpha-chain with full length variable region and truncated constant region containing cysteine substitution.
MSLSSLLKVVTASLWLGPGIAQKITQTQPGMFVQEKEAVTLDCTYDTSDQSYGLFWYKQPSSGEMIFLIYQGSYDEQNATEGRYSLNFQKARKSANLVISASQLGDSAMYFCAMREIYSSASKIIFGSGTRLSIRPNIQNPDPAVYQLRDSKSSDKSVCLFTDFDSQTNVSQSKDSDVYITDKCVLDMRSMDFKSNSAVAWSNKSDFACANAFNNSIIPEDTFFPSPESSC

SEQ ID NO: 25 - protein, 264 aa, Artificial Sequence
  Soluble hTERT-TCR-1 beta-chain with truncated variable region and truncated constant region containing cysteine substitution.
MGTRLLFWVAFCLLGADHTVSQSPSNKVTEKGKDVELRCDPISGHTALYWYRQSLGQGLEFLIYFQGNSAPDKSGLPSDRFSAERTGGSVSTLTIQRTQQEDSAVYLCASSLGGGDHTDTQYFGPGTRLTVLEDLKNVFPPEVAVFEPSEAEISHTQKATLVCLATGFYPDHVELSWWVNGKEVHSGVCTDPQPLKEQPALNDSRYCLSSRLRVSATFWQNPRNHFRCQVQFYGLSENDEWTQDRAKPVTQIVSAEAWGRADCG

SEQ ID NO: 26 - protein, 267 aa, Artificial Sequence
  Soluble hTERT-TCR-1 beta-chain with full-length variable region and truncated constant region containing cysteine substitution.
MGTRLLFWVAFCLLGADHTGAGVSQSPSNKVTEKGKDVELRCDPISGHTALYWYRQSLGQGLEFLIYFQGNSAPDKSGLPSDRFSAERTGGSVSTLTIQRTQQEDSAVYLCASSLGGGDHTDTQYFGPGTRLTVLEDLKNVFPPEVAVFEPSEAEISHTQKATLVCLATGFYPDHVELSWWVNGKEVHSGVCTDPQPLKEQPALNDSRYCLSSRLRVSATFWQNPRNHFRCQVQFYGLSENDEWTQDRAKPVTQIVSAEAWGRADCG

SEQ ID NO: 27 - protein, 518 aa, Artificial Sequence
  Soluble hTERT-TCR-1 scTCR with truncated variable regions.
MSLSSLLKVVTASLWLGPGIITQTQPGMFVQEKEAVTLDCTYDTSDQSYGLFWYKQPSSGEMIFLIYQGSYDEQNATEGRYSLNFQKARKSANLVISASQLGDSAMYFCAMREIYSSASKIIFGSGTRLSIRPNIQNPDPAVYQLRDSKSSDKSVCLFTDFDSQTNVSQSKDSDVYITDKCVLDMRSMDFKSNSAVAWSNKSDFACANAFNNSIIPEDTFFPSPESSCRAKRGSGATNFSLLKQAGDVEENPGPMGTRLLFWVAFCLLGADHTVSQSPSNKVTEKGKDVELRCDPISGHTALYWYRQSLGQGLEFLIYFQGNSAPDKSGLPSDRFSAERTGGSVSTLTIQRTQQEDSAVYLCASSLGGGDHTDTQYFGPGTRLTVLEDLKNVFPPEVAVFEPSEAEISHTQKATLVCLATGFYPDHVELSWWVNGKEVHSGVCTDPQPLKEQPALNDSRYCLSSRLRVSATFWQNPRNHFRCQVQFYGLSENDEWTQDRAKPVTQIVSAEAWGRADCG

SEQ ID NO: 28 - protein, 524 aa, Artificial Sequence
  Soluble hTERT-TCR-1 scTCR with full-length variable regions.
MSLSSLLKVVTASLWLGPGIAQKITQTQPGMFVQEKEAVTLDCTYDTSDQSYGLFWYKQPSSGEMIFLIYQGSYDEQNATEGRYSLNFQKARKSANLVISASQLGDSAMYFCAMREIYSSASKIIFGSGTRLSIRPNIQNPDPAVYQLRDSKSSDKSVCLFTDFDSQTNVSQSKDSDVYITDKCVLDMRSMDFKSNSAVAWSNKSDFACANAFNNSIIPEDTFFPSPESSCRAKRGSGATNFSLLKQAGDVEENPGPMGTRLLFWVAFCLLGADHTGAGVSQSPSNKVTEKGKDVELRCDPISGHTALYWYRQSLGQGLEFLIYFQGNSAPDKSGLPSDRFSAERTGGSVSTLTIQRTQQEDSAVYLCASSLGGGDHTDTQYFGPGTRLTVLEDLKNVFPPEVAVFEPSEAEISHTQKATLVCLATGFYPDHVELSWWVNGKEVHSGVCTDPQPLKEQPALNDSRYCLSSRLRVSATFWQNPRNHFRCQVQFYGLSENDEWTQDRAKPVTQIVSAEAWGRADCG

SEQ ID NO: 29 - protein, 96 aa, Homo sapiens
PNIQNPDPAVYQLRDSKSSDKSVCLFTDFDSQTNVSQSKDSDVYITDKTVLDMRSMDFKSNSAVAWSNKSDFACANAFNNSIIPEDTFFPSPESSC

SEQ ID NO: 30 - protein, 132 aa, Homo sapiens
EDLKNVFPPEVAVFEPSEAEISHTQKATLVCLATGFYPDHVELSWWVNGKEVHSGVSTDPQPLKEQPALNDSRYCLSSRLRVSATFWQNPRNHFRCQVQFYGLSENDEWTQDRAKPVTQIVSAEAWGRADCG

SEQ ID NO: 31 - protein, 20 aa, Homo sapiens
MSLSSLLKVVTASLWLGPGI

SEQ ID NO: 32 - protein, 19 aa, Homo sapiens
MGTRLLFWVAFCLLGADHT

SEQ ID NO: 33 - protein, 233 aa, Artificial Sequence
  Mature soluble hTERT-TCR-1 alpha-chain with truncated variable region, cysteine-substituted constant region and residual 2A amino acids at C-terminus.
ITQTQPGMFVQEKEAVTLDCTYDTSDQSYGLFWYKQPSSGEMIFLIYQGSYDEQNATEGRYSLNFQKARKSANLVISASQLGDSAMYFCAMREIYSSASKIIFGSGTRLSIRPNIQNPDPAVYQLRDSKSSDKSVCLFTDFDSQTNVSQSKDSDVYITDKCVLDMRSMDFKSNSAVAWSNKSDFACANAFNNSIIPEDTFFPSPESSCRAKRGSGATNFSLLKQAGDVEENPG

SEQ ID NO: 34 - protein, 236 aa, Artificial Sequence
  Mature soluble hTERT-TCR-1 alpha-chain with full-length variable region, cysteine-substituted constant region and residual 2A amino acids at C-terminus.
AQKITQTQPGMFVQEKEAVTLDCTYDTSDQSYGLFWYKQPSSGEMIFLIYQGSYDEQNATEGRYSLNFQKARKSANLVISASQLGDSAMYFCAMREIYSSASKIIFGSGTRLSIRPNIQNPDPAVYQLRDSKSSDKSVCLFTDFDSQTNVSQSKDSDVYITDKCVLDMRSMDFKSNSAVAWSNKSDFACANAFNNSIIPEDTFFPSPESSCRAKRGSGATNFSLLKQAGDVEENPG

SEQ ID NO: 35 - protein, 270 aa, Artificial Sequence
  Mature soluble hTERT-TCR-1 beta-chain with truncated variable region, cysteine-substituted constant region and residual 2A amino acids at C-terminus.
VSQSPSNKVTEKGKDVELRCDPISGHTALYWYRQSLGQGLEFLIYFQGNSAPDKSGLPSDRFSAERTGGSVSTLTIQRTQQEDSAVYLCASSLGGGDHTDTQYFGPGTRLTVLEDLKNVFPPEVAVFEPSEAEISHTQKATLVCLATGFYPDHVELSWWVNGKEVHSGVCTDPQPLKEQPALNDSRYCLSSRLRVSATFWQNPRNHFRCQVQFYGLSENDEWTQDRAKPVTQIVSAEAWGRADCGRAKRGSGATNFSLLKQAGDVEENPG

SEQ ID NO: 36 - protein, 273 aa, Artificial Sequence
  Mature soluble hTERT-TCR-1 beta-chain with full-length variable region, cysteine-substituted constant region and residual 2A amino acids at C-terminus.
GAGVSQSPSNKVTEKGKDVELRCDPISGHTALYWYRQSLGQGLEFLIYFQGNSAPDKSGLPSDRFSAERTGGSVSTLTIQRTQQEDSAVYLCASSLGGGDHTDTQYFGPGTRLTVLEDLKNVFPPEVAVFEPSEAEISHTQKATLVCLATGFYPDHVELSWWVNGKEVHSGVCTDPQPLKEQPALNDSRYCLSSRLRVSATFWQNPRNHFRCQVQFYGLSENDEWTQDRAKPVTQIVSAEAWGRADCGRAKRGSGATNFSLLKQAGDVEENPG

SEQ ID NO: 37 - protein, 254 aa, Homo sapiens
ITQTQPGMFVQEKEAVTLDCTYDTSDQSYGLFWYKQPSSGEMIFLIYQGSYDEQNATEGRYSLNFQKARKSANLVISASQLGDSAMYFCAMREIYSSASKIIFGSGTRLSIRPNIQNPDPAVYQLRDSKSSDKSVCLFTDFDSQTNVSQSKDSDVYITDKTVLDMRSMDFKSNSAVAWSNKSDFACANAFNNSIIPEDTFFPSPESSCDVKLVEKSFETDTNLNFQNLSVIGFRILLLKVAGFNLLMTLRLWSS

SEQ ID NO: 38 - protein, 257 aa, Homo sapiens
AQKITQTQPGMFVQEKEAVTLDCTYDTSDQSYGLFWYKQPSSGEMIFLIYQGSYDEQNATEGRYSLNFQKARKSANLVISASQLGDSAMYFCAMREIYSSASKIIFGSGTRLSIRPNIQNPDPAVYQLRDSKSSDKSVCLFTDFDSQTNVSQSKDSDVYITDKTVLDMRSMDFKSNSAVAWSNKSDFACANAFNNSIIPEDTFFPSPESSCDVKLVEKSFETDTNLNFQNLSVIGFRILLLKVAGFNLLMTLRLWSS

SEQ ID NO: 39 - protein, 292 aa, Homo sapiens
VSQSPSNKVTEKGKDVELRCDPISGHTALYWYRQSLGQGLEFLIYFQGNSAPDKSGLPSDRFSAERTGGSVSTLTIQRTQQEDSAVYLCASSLGGGDHTDTQYFGPGTRLTVLEDLKNVFPPEVAVFEPSEAEISHTQKATLVCLATGFYPDHVELSWWVNGKEVHSGVSTDPQPLKEQPALNDSRYCLSSRLRVSATFWQNPRNHFRCQVQFYGLSENDEWTQDRAKPVTQIVSAEAWGRADCGFTSESYQQGVLSATILYEILLGKATLYAVLVSALVLMAMVKRKDSRG

SEQ ID NO: 40 - protein, 295 aa, Homo sapiens
GAGVSQSPSNKVTEKGKDVELRCDPISGHTALYWYRQSLGQGLEFLIYFQGNSAPDKSGLPSDRFSAERTGGSVSTLTIQRTQQEDSAVYLCASSLGGGDHTDTQYFGPGTRLTVLEDLKNVFPPEVAVFEPSEAEISHTQKATLVCLATGFYPDHVELSWWVNGKEVHSGVSTDPQPLKEQPALNDSRYCLSSRLRVSATFWQNPRNHFRCQVQFYGLSENDEWTQDRAKPVTQIVSAEAWGRADCGFTSESYQQGVLSATILYEILLGKATLYAVLVSALVLMAMVKRKDSRG

SEQ ID NO: 41 - protein, 208 aa, Artificial Sequence
  Mature soluble hTERT-TCR-1 alpha-chain with truncated variable region and cysteine-substituted constant region.
ITQTQPGMFVQEKEAVTLDCTYDTSDQSYGLFWYKQPSSGEMIFLIYQGSYDEQNATEGRYSLNFQKARKSANLVISASQLGDSAMYFCAMREIYSSASKIIFGSGTRLSIRPNIQNPDPAVYQLRDSKSSDKSVCLFTDFDSQTNVSQSKDSDVYITDKCVLDMRSMDFKSNSAVAWSNKSDFACANAFNNSIIPEDTFFPSPESSC

SEQ ID NO: 42 - protein, 211 aa, Artificial Sequence
  Mature soluble hTERT-TCR-1 alpha-chain with full-length variable region and cysteine-substituted constant region.
AQKITQTQPGMFVQEKEAVTLDCTYDTSDQSYGLFWYKQPSSGEMIFLIYQGSYDEQNATEGRYSLNFQKARKSANLVISASQLGDSAMYFCAMREIYSSASKIIFGSGTRLSIRPNIQNPDPAVYQLRDSKSSDKSVCLFTDFDSQTNVSQSKDSDVYITDKCVLDMRSMDFKSNSAVAWSNKSDFACANAFNNSIIPEDTFFPSPESSC

SEQ ID NO: 43 - protein, 245 aa, Artificial Sequence
  Mature soluble hTERT-TCR-1 beta-chain with truncated variable region and cysteine-substituted constant region.
VSQSPSNKVTEKGKDVELRCDPISGHTALYWYRQSLGQGLEFLIYFQGNSAPDKSGLPSDRFSAERTGGSVSTLTIQRTQQEDSAVYLCASSLGGGDHTDTQYFGPGTRLTVLEDLKNVFPPEVAVFEPSEAEISHTQKATLVCLATGFYPDHVELSWWVNGKEVHSGVCTDPQPLKEQPALNDSRYCLSSRLRVSATFWQNPRNHFRCQVQFYGLSENDEWTQDRAKPVTQIVSAEAWGRADCG

SEQ ID NO: 44 - protein, 248 aa, Artificial Sequence
  Mature soluble hTERT-TCR-1 beta-chain with full-length variable region and cysteine-substituted constant region.
GAGVSQSPSNKVTEKGKDVELRCDPISGHTALYWYRQSLGQGLEFLIYFQGNSAPDKSGLPSDRFSAERTGGSVSTLTIQRTQQEDSAVYLCASSLGGGDHTDTQYFGPGTRLTVLEDLKNVFPPEVAVFEPSEAEISHTQKATLVCLATGFYPDHVELSWWVNGKEVHSGVCTDPQPLKEQPALNDSRYCLSSRLRVSATFWQNPRNHFRCQVQFYGLSENDEWTQDRAKPVTQIVSAEAWGRADCG

SEQ ID NO: 45 - protein, 27 aa, Homo sapiens
FWVLVVVGGVLACYSLLVTVAFIIFWV

SEQ ID NO: 46 - protein, 112 aa, Homo sapiens
RVKFSRSADAPAYQQGQNQLYNELNLGRREEYDVLDKRRGRDPEMGGKPRRKNPQEGLYNELQKDKMAEAYSEIGMKGERRRGKGHDGLYQGLSTATKDTYDALHMQALPPR

SEQ ID NO: 47 - protein, 391 aa, Artificial Sequence
  Mature soluble hTERT-TCR-1 alpha-chain with full-length variable region, cysteine-substituted constant region and CD28-CD3zeta tail.
AQKITQTQPGMFVQEKEAVTLDCTYDTSDQSYGLFWYKQPSSGEMIFLIYQGSYDEQNATEGRYSLNFQKARKSANLVISASQLGDSAMYFCAMREIYSSASKIIFGSGTRLSIRPNIQNPDPAVYQLRDSKSSDKSVCLFTDFDSQTNVSQSKDSDVYITDKCVLDMRSMDFKSNSAVAWSNKSDFACANAFNNSIIPEDTFFPSPESSCFWVLVVVGGVLACYSLLVTVAFIIFWVRSKRSRLLHSDYMNMTPRRPGPTRKHYQPYAPPRDFAAYRSRVKFSRSADAPAYQQGQNQLYNELNLGRREEYDVLDKRRGRDPEMGGKPRRKNPQEGLYNELQKDKMAEAYSEIGMKGERRRGKGHDGLYQGLSTATKDTYDALHMQALPPR

SEQ ID NO: 48 - protein, 428 aa, Artificial Sequence
  Mature soluble hTERT-TCR-1 beta-chain with full-length variable region, cysteine-substituted constant region and CD28-CD3zeta tail.
GAGVSQSPSNKVTEKGKDVELRCDPISGHTALYWYRQSLGQGLEFLIYFQGNSAPDKSGLPSDRFSAERTGGSVSTLTIQRTQQEDSAVYLCASSLGGGDHTDTQYFGPGTRLTVLEDLKNVFPPEVAVFEPSEAEISHTQKATLVCLATGFYPDHVELSWWVNGKEVHSGVCTDPQPLKEQPALNDSRYCLSSRLRVSATFWQNPRNHFRCQVQFYGLSENDEWTQDRAKPVTQIVSAEAWGRADCGFWVLVVVGGVLACYSLLVTVAFIIFWVRSKRSRLLHSDYMNMTPRRPGPTRKHYQPYAPPRDFAAYRSRVKFSRSADAPAYQQGQNQLYNELNLGRREEYDVLDKRRGRDPEMGGKPRRKNPQEGLYNELQKDKMAEAYSEIGMKGERRRGKGHDGLYQGLSTATKDTYDALHMQALPPR

SEQ ID NO: 49 - protein, 704 aa, Artificial Sequence
  hTERT-TCR-1 scTCR-CAR with CD28-CD3zeta tail on alpha-chain
MSLSSLLKVVTASLWLGPGIAQKITQTQPGMFVQEKEAVTLDCTYDTSDQSYGLFWYKQPSSGEMIFLIYQGSYDEQNATEGRYSLNFQKARKSANLVISASQLGDSAMYFCAMREIYSSASKIIFGSGTRLSIRPNIQNPDPAVYQLRDSKSSDKSVCLFTDFDSQTNVSQSKDSDVYITDKCVLDMRSMDFKSNSAVAWSNKSDFACANAFNNSIIPEDTFFPSPESSCFWVLVVVGGVLACYSLLVTVAFIIFWVRSKRSRLLHSDYMNMTPRRPGPTRKHYQPYAPPRDFAAYRSRVKFSRSADAPAYQQGQNQLYNELNLGRREEYDVLDKRRGRDPEMGGKPRRKNPQEGLYNELQKDKMAEAYSEIGMKGERRRGKGHDGLYQGLSTATKDTYDALHMQALPPRRAKRGSGATNFSLLKQAGDVEENPGPMGTRLLFWVAFCLLGADHTGAGVSQSPSNKVTEKGKDVELRCDPISGHTALYWYRQSLGQGLEFLIYFQGNSAPDKSGLPSDRFSAERTGGSVSTLTIQRTQQEDSAVYLCASSLGGGDHTDTQYFGPGTRLTVLEDLKNVFPPEVAVFEPSEAEISHTQKATLVCLATGFYPDHVELSWWVNGKEVHSGVCTDPQPLKEQPALNDSRYCLSSRLRVSATFWQNPRNHFRCQVQFYGLSENDEWTQDRAKPVTQIVSAEAWGRADCG

SEQ ID NO: 50 - protein, 704 aa, Artificial Sequence
  hTERT-TCR-1 scTCR-CAR with CD28-CD3zeta tail on beta-chain.
MSLSSLLKVVTASLWLGPGIAQKITQTQPGMFVQEKEAVTLDCTYDTSDQSYGLFWYKQPSSGEMIFLIYQGSYDEQNATEGRYSLNFQKARKSANLVISASQLGDSAMYFCAMREIYSSASKIIFGSGTRLSIRPNIQNPDPAVYQLRDSKSSDKSVCLFTDFDSQTNVSQSKDSDVYITDKCVLDMRSMDFKSNSAVAWSNKSDFACANAFNNSIIPEDTFFPSPESSCRAKRGSGATNFSLLKQAGDVEENPGPMGTRLLFWVAFCLLGADHTGAGVSQSPSNKVTEKGKDVELRCDPISGHTALYWYRQSLGQGLEFLIYFQGNSAPDKSGLPSDRFSAERTGGSVSTLTIQRTQQEDSAVYLCASSLGGGDHTDTQYFGPGTRLTVLEDLKNVFPPEVAVFEPSEAEISHTQKATLVCLATGFYPDHVELSWWVNGKEVHSGVCTDPQPLKEQPALNDSRYCLSSRLRVSATFWQNPRNHFRCQVQFYGLSENDEWTQDRAKPVTQIVSAEAWGRADCGFWVLVVVGGVLACYSLLVTVAFIIFWVRSKRSRLLHSDYMNMTPRRPGPTRKHYQPYAPPRDFAAYRSRVKFSRSADAPAYQQGQNQLYNELNLGRREEYDVLDKRRGRDPEMGGKPRRKNPQEGLYNELQKDKMAEAYSEIGMKGERRRGKGHDGLYQGLSTATKDTYDALHMQALPPR

SEQ ID NO: 51 - protein, 1132 aa, Homo sapiens
MPRAPRCRAVRSLLRSHYREVLPLATFVRRLGPQGWRLVQRGDPAAFRALVAQCLVCVPWDARPPPAAPSFRQVSCLKELVARVLQRLCERGAKNVLAFGFALLDGARGGPPEAFTTSVRSYLPNTVTDALRGSGAWGLLLRRVGDDVLVHLLARCALFVLVAPSCAYQVCGPPLYQLGAATQARPPPHASGPRRRLGCERAWNHSVREAGVPLGLPAPGARRRGGSASRSLPLPKRPRRGAAPEPERTPVGQGSWAHPGRTRGPSDRGFCVVSPARPAEEATSLEGALSGTRHSHPSVGRQHHAGPPSTSRPPRPWDTPCPPVYAETKHFLYSSGDKEQLRPSFLLSSLRPSLTGARRLVETIFLGSRPWMPGTPRRLPRLPQRYWQMRPLFLELLGNHAQCPYGVLLKTHCPLRAAVTPAAGVCAREKPQGSVAAPEEEDTDPRRLVQLLRQHSSPWQVYGFVRACLRRLVPPGLWGSRHNERRFLRNTKKFISLGKHAKLSLQELTWKMSVRDCAWLRRSPGVGCVPAAEHRLREEILAKFLHWLMSVYVVELLRSFFYVTETTFQKNRLFFYRKSVWSKLQSIGIRQHLKRVQLRELSEAEVRQHREARPALLTSRLRFIPKPDGLRPIVNMDYVVGARTFRREKRAERLTSRVKALFSVLNYERARRPGLLGASVLGLDDIHRAWRTFVLRVRAQDPPPELYFVKVDVTGAYDTIPQDRLTEVIASIIKPQNTYCVRRYAVVQKAAHGHVRKAFKSHVSTLTDLQPYMRQFVAHLQETSPLRDAVVIEQSSSLNEASSGLFDVFLRFMCHHAVRIRGKSYVQCQGIPQGSILSTLLCSLCYGDMENKLFAGIRRDGLLLRLVDDFLLVTPHLTHAKTFLRTLVRGVPEYGCVVNLRKTVVNFPVEDEALGGTAFVQMPAHGLFPWCGLLLDTRTLEVQSDYSSYARTSIRASLTFNRGFKAGRNMRRKLFGVLRLKCHSLFLDLQVNSLQTVCTNIYKILLLQAYRFHACVLQLPFHQQVWKNPTFFLRVISDTASLCYSILKAKNAGMSLGAKGAAGPLPSEAVQWLCHQAFLLKLTRHRVTYVPLLGSLRTAQTQLSRKLPGTTLTALEAAANPALPSDFKTILD

SEQ ID NO: 52 - protein, 16 aa, Homo sapiens
EARPALLTSRLRFIPK

SEQ ID NO: 53 - protein, 8 aa, Picornaviridae
  X (2)..(2): Valine or Isoleucine
  X (4)..(4): Any amino acid
DXEXNPGP

SEQ ID NO: 54 - protein, 208 aa, Artificial Sequence
  Mature soluble hTERT-TCR-1 alpha-chain with truncated variable region.
ITQTQPGMFVQEKEAVTLDCTYDTSDQSYGLFWYKQPSSGEMIFLIYQGSYDEQNATEGRYSLNFQKARKSANLVISASQLGDSAMYFCAMREIYSSASKIIFGSGTRLSIRPNIQNPDPAVYQLRDSKSSDKSVCLFTDFDSQTNVSQSKDSDVYITDKTVLDMRSMDFKSNSAVAWSNKSDFACANAFNNSIIPEDTFFPSPESSC

SEQ ID NO: 55 - protein, 211 aa, Homo sapiens
AQKITQTQPGMFVQEKEAVTLDCTYDTSDQSYGLFWYKQPSSGEMIFLIYQGSYDEQNATEGRYSLNFQKARKSANLVISASQLGDSAMYFCAMREIYSSASKIIFGSGTRLSIRPNIQNPDPAVYQLRDSKSSDKSVCLFTDFDSQTNVSQSKDSDVYITDKTVLDMRSMDFKSNSAVAWSNKSDFACANAFNNSIIPEDTFFPSPESSC

SEQ ID NO: 56 - protein, 245 aa, Artificial Sequence
  Mature soluble hTERT-TCR-1 beta-chain with truncated variable region.
VSQSPSNKVTEKGKDVELRCDPISGHTALYWYRQSLGQGLEFLIYFQGNSAPDKSGLPSDRFSAERTGGSVSTLTIQRTQQEDSAVYLCASSLGGGDHTDTQYFGPGTRLTVLEDLKNVFPPEVAVFEPSEAEISHTQKATLVCLATGFYPDHVELSWWVNGKEVHSGVSTDPQPLKEQPALNDSRYCLSSRLRVSATFWQNPRNHFRCQVQFYGLSENDEWTQDRAKPVTQIVSAEAWGRADCG

SEQ ID NO: 57 - protein, 248 aa, Homo sapiens
GAGVSQSPSNKVTEKGKDVELRCDPISGHTALYWYRQSLGQGLEFLIYFQGNSAPDKSGLPSDRFSAERTGGSVSTLTIQRTQQEDSAVYLCASSLGGGDHTDTQYFGPGTRLTVLEDLKNVFPPEVAVFEPSEAEISHTQKATLVCLATGFYPDHVELSWWVNGKEVHSGVSTDPQPLKEQPALNDSRYCLSSRLRVSATFWQNPRNHFRCQVQFYGLSENDEWTQDRAKPVTQIVSAEAWGRADCG

SEQ ID NO: 58 - protein, 41 aa, Homo sapiens
RSKRSRLLHSDYMNMTPRRPGPTRKHYQPYAPPRDFAAYRS

SEQ ID NO: 59 - protein, 180 aa, Artificial Sequence
  CD28 transmembrane domain - CD28 intracellular domain - CD3zeta intracellular domain CAR signalling tail
FWVLVVVGGVLACYSLLVTVAFIIFWVRSKRSRLLHSDYMNMTPRRPGPTRKHYQPYAPPRDFAAYRSRVKFSRSADAPAYQQGQNQLYNELNLGRREEYDVLDKRRGRDPEMGGKPRRKNPQEGLYNELQKDKMAEAYSEIGMKGERRRGKGHDGLYQGLSTATKDTYDALHMQALPPR

SEQ ID NO: 60 - protein, 411 aa, Artificial Sequence
  Mature soluble hTERT-TCR-1 alpha-chain with full-length variable region, cysteine-substituted constant region and CD28-CD3zeta tail, and leader sequence.
MSLSSLLKVVTASLWLGPGIAQKITQTQPGMFVQEKEAVTLDCTYDTSDQSYGLFWYKQPSSGEMIFLIYQGSYDEQNATEGRYSLNFQKARKSANLVISASQLGDSAMYFCAMREIYSSASKIIFGSGTRLSIRPNIQNPDPAVYQLRDSKSSDKSVCLFTDFDSQTNVSQSKDSDVYITDKCVLDMRSMDFKSNSAVAWSNKSDFACANAFNNSIIPEDTFFPSPESSCFWVLVVVGGVLACYSLLVTVAFIIFWVRSKRSRLLHSDYMNMTPRRPGPTRKHYQPYAPPRDFAAYRSRVKFSRSADAPAYQQGQNQLYNELNLGRREEYDVLDKRRGRDPEMGGKPRRKNPQEGLYNELQKDKMAEAYSEIGMKGERRRGKGHDGLYQGLSTATKDTYDALHMQALPPR

SEQ ID NO: 61 - protein, 447 aa, Artificial Sequence
  Mature soluble hTERT-TCR-1 beta-chain with full-length variable region, cysteine-substituted constant region and CD28-CD3zeta tail, and leader sequence.
MGTRLLFWVAFCLLGADHTGAGVSQSPSNKVTEKGKDVELRCDPISGHTALYWYRQSLGQGLEFLIYFQGNSAPDKSGLPSDRFSAERTGGSVSTLTIQRTQQEDSAVYLCASSLGGGDHTDTQYFGPGTRLTVLEDLKNVFPPEVAVFEPSEAEISHTQKATLVCLATGFYPDHVELSWWVNGKEVHSGVCTDPQPLKEQPALNDSRYCLSSRLRVSATFWQNPRNHFRCQVQFYGLSENDEWTQDRAKPVTQIVSAEAWGRADCGFWVLVVVGGVLACYSLLVTVAFIIFWVRSKRSRLLHSDYMNMTPRRPGPTRKHYQPYAPPRDFAAYRSRVKFSRSADAPAYQQGQNQLYNELNLGRREEYDVLDKRRGRDPEMGGKPRRKNPQEGLYNELQKDKMAEAYSEIGMKGERRRGKGHDGLYQGLSTATKDTYDALHMQALPPR

SEQ ID NO: 62 - DNA, 834 bp, Homo sapiens
atgtcactttctagcctgctgaaggtggtcacagcttcactgtggctaggacctggcattgcccagaagataactcaaacccaaccaggaatgttcgtgcaggaaaaggaggctgtgactctggactgcacatatgacaccagtgatcaaagttatggtctattctggtacaagcagcccagcagtggggaaatgatttttcttatttatcaggggtcttatgacgagcaaaatgcaacagaaggtcgctactcattgaatttccagaaggcaagaaaatccgccaaccttgtcatctccgcttcacaactgggggactcagcaatgtatttctgtgcaatgagagagatctacagcagtgcttccaagataatctttggatcagggaccagactcagcatccggccaaatatccagaaccctgaccctgccgtgtaccagctgagagactctaaatccagtgacaagtctgtctgcctattcaccgattttgattctcaaacaaatgtgtcacaaagtaaggattctgatgtgtatatcacagacaaaactgtgctagacatgaggtctatggacttcaagagcaacagtgctgtggcctggagcaacaaatctgactttgcatgtgcaaacgccttcaacaacagcattattccagaagacaccttcttccccagcccagaaagttcctgtgatgtcaagctggtcgagaaaagctttgaaacagatacgaacctaaactttcaaaacctgtcagtgattgggttccgaatcctcctcctgaaagtggccgggtttaatctgctcatgacgctgcggctgtggtccagctag

SEQ ID NO: 63 - DNA, 834 bp, Homo sapiens; identical to SEQ ID NO: 62

SEQ ID NO: 64 - DNA, 78 bp, Picornaviridae
agagccaagagaggcagcggcgccaccaacttcagcctgctgaagcaggccggcgacgtggaagagaaccctggacca

SEQ ID NO: 65 - protein, 15 aa, Escherichia coli
GGLNDIFEAQKIEWH

SEQ ID NO: 66 - protein, 25 aa, Picornaviridae
RAKRGSGATNFSLLKQAGDVEENPG

SEQ ID NO: 67 - protein, 5 aa, Artificial Sequence
  G4S linker unit
GGGGS

SEQ ID NO: 68 - protein, 1048 aa, Artificial Sequence
  68
MDDQRDLISNNEQLPMLGRRPGAPESKCSRGALYTGFSILVTLLLAGQATTAYFLYQQQGRLDKLTVTSQNLQLENLRMKLPKPPKPVSKGTEARPALLTSRLRFIPKLEQNATKYGNMTEDHVMHLLQNADPLKVYPPLKGSFPENLRHLKNTMETIDWKVFESWMHHWLLFEMSRHSLEQKPTDAPPKESLELEDPSSGLGVTKQDLGPVPMEFRAKRGSGATNFSLLKQAGDVEENPGPMEDAKNIKKGPAPFYPLEDGTAGEQLHKAMKRYALVPGTIAFTDAHIEVDITYAEYFEMSVRLAEAMKRYGLNTNHRIVVCSENSLQFFMPVLGALFIGVAVAPANDIYNERELLNSMGISQPTVVFVSKKGLQKILNVQKKLPIIQKIIIMDSKTDYQGFQSMYTFVTSHLPPGFNEYDFVPESFDRDKTIALIMNSSGSTGLPKGVALPHRTACVRFSHARDPIFGNQIIPDTAILSVVPFHHGFGMFTTLGYLICGFRVVLMYRFEEELFLRSLQDYKIQSALLVPTLFSFFAKSTLIDKYDLSNLHEIASGGAPLSKEVGEAVAKRFHLPGIRQGYGLTETTSAILITPEGDDKPGAVGKVVPFFEAKVVDLDTGKTLGVNQRGELCVRGPMIMSGYVNNPEATNALIDKDGWLHSGDIAYWDEDEHFFIVDRLKSLIKYKGYQVAPAELESILLQHPNIFDAGVAGLPDDDAGELPAAVVVLEHGKTMTEKEIVDYVASQVTTAKKLRGGVVFVDEVPKGLTGKLDARKIREILIKAKKGGKIAVAKGKSEEELANCFRIPPLVSKGEELFTGVVPILVELDGDVNGHKFSVSGEGEGDATYGKLTLKFICTTGKLPVPWPTLVTTLTYGVQCFSRYPDHMKQHDFFKSAMPEGYVQERTIFFKDDGNYKTRAEVKFEGDTLVNRIELKGIDFKEDGNILGHKLEYNYNSHNVYIMADKQKNGIKVNFKIRHNIEDGSVQLADHYQQNTPIGDGPVLLPDNHYLSTQSALSKDPNEKRDHMVLLEFVTAAGITLGMDELYK